European Patent Application EP 4 438 714 A1, published October 2, 2024. Title: ACID-RESISTANT YEAST STRAIN FOR HIGH-YIELD PRODUCTION OF L-MALIC ACID, AND CONSTRUCTION METHOD THEREFOR AND USE THEREOF. Applicant: Tianjin Institute of Industrial Biotechnology, Chinese Academy of Sciences. The sequence listing filed with the application follows.

SEQUENCE LISTING (115 sequences)

SEQ ID NO: 1 - DNA, 1339 bp, Sorghum bicolor
  source 1..1339: mol_type = other DNA
actaccacccccaacacaaacacaatgggtttgtctaccgcatactctccagttggttctcacttggctccagcaccattaggtcacagaagatccgctcaattacatagaccaagaagagcattgttagctaccgttagatgttccgttgatgctgcaaagcaagttcaagatggtgttgctactgcagaagctccagcaactagaaaggattctttcggtgttttctctactacctacgacttaaaggcagaagataagaccaagtcctggaagaagttggttaacattgctgtttctggtgcagctggtatgatttccaaccacttgttattcaagttggcttctggtgaagttttcggtcaagaccaaccaattgcattaaagttattgggttccgaaagatctttccaagctttggaaggtgttgctatggaattggaagattccttgtacccattattgagagaagtttccattggtattgacccatacgaagttttcgaagacgttgattgggcattattgattggtgctaagccaagaggtccaggtatggaaagagcagctttgttagacattaacggtcaaattttcgctgatcaaggtaaggcattgaacgctgttgcatctaagaacgttaaggttttggttgttggtaacccatgtaacaccaacgctttgatttgtttgaagaacgcaccagatattccagctaagaacttccacgcattaaccagattggacgaaaacagagcaaagtgtcaattggctttaaaggcaggtgttttctacgataaggtttccaacgttaccatttggggtaaccactctactacccaagttccagatttcttgaacgcaaagattgacggtagaccagttaaggaagttattaaggacactaagtggttggaagaagaattcaccattactgttcaaaagagaggtggtgctttgattcaaaagtggggtagatcctctgcagcttccaccgctgtttctattgctgacgcaattaagtccttggttaccccaactccagaaggtgactggttttccaccggtgtttacaccactggtaacccatacggtattgcagaagacattgttttctccatgccatgtagatctaagggtgatggtgactacgaattggcaaccgatgtttccatggacgatttcttatgggaaagaattaagaagtccgaagcagaattgttggcagaaaagaaggctgttgctcacttgaccggtgaaggtaacgcatactgtgacgttccagaagatactatgttgccaggtgaagtttaactacaacaagatgtttgttcaaggg

SEQ ID NO: 2 - DNA, 1373 bp, Schizosaccharomyces pombe
  source 1..1373: mol_type = other DNA
caaaacacacaaacaaacacaattacaaaaaatgggtgaattaaaggaaatcttaaagcaaagataccacgaattattggactggaatgtcaaggcaccacacgtcccattgtctcaaagattaaagcactttacttggtcttggttcgcttgtactatggcaaccggtggtgttggtttgattattggttccttcccattcagattctacggtttaaacaccatcggtaaaatcgtttacatcttgcaaattttcttgttctctttgtttggttcctgtatgttgttcagattcattaagtacccatctactattaaggattcctggaaccaccacttggaaaagttgtttattgcaacttgtttgttgtctatttccaccttcattgatatgttggctatctacgcatacccagacactggtgaatggatggtttgggttattagaatcttgtactacatctacgttgctgtttctttcatctactgtgttatggctttctttaccattttcaacaaccacgtttacactattgaaaccgcttctccagcatggattttaccaattttcccaccaatgatttgtggtgttattgctggtgcagttaactccactcaaccagctcatcaattgaagaacatggttattttcggtatcttgttccaaggtttgggtttttgggtttacttgttattgttcgcagttaacgttttaagattctttaccgttggtttggctaagccacaagacagaccaggtatgtttatgttcgttggtccaccagctttttctggtttagcattgattaacattgctagaggtgcaatgggttccagaccatacattttcgttggtgcaaactcttccgaatacttaggtttcgtttctacttttatggctattttcatttggggtttggctgcatggtgttactgtttagcaatggtttcctttttggctggtttctttactagagctccattgaagttcgcatgtggttggtttgctttcattttcccaaacgttggtttcgttaactgtaccatcgaaatcggtaaaatgatcgattctaaggcattccaaatgttcggtcacatcatcggtgttattttgtgtatccaatggatcttgttgatgtacttgatggttagagcatttttagttaacgacttgtgttaccctggtaaagatgaagacgctcacccaccaccaaagccaaacactggtgttttaaacccaaccttcccaccagaaaaggctccagcatccttggaaaaggttgatacccacgttacctctactggtggtgaatctgacccaccatcctctgaacacgaatccgtctaaatcactttctgtcaattgtcttaat

SEQ ID NO: 3 - DNA, 1763 bp, Schizosaccharomyces pombe
  source 1..1763: mol_type = other DNA
caaaacacacaaacaaacacaattacaaaaaatggcatccgaatggccagaaacctccagagcatcctccgttgaagaaaacccaaagttgaacatcccagaaatcgttgaatccgtctctgactccaagccatctttaaagaaccaattctccactaccgttattgattcttccgacttgaacgtttttaacgatggtgctgaaactaccgttaaggaacaagaattcacttcttccgaattgagaagattgcaaaagttgagattgaagatggacttgagaatcatcccatgtttgtggatcttgtactttttgtcttgttgtttgagattcactgtttctttgtcctttactatgaacaccgctcaaggtcactccttaattcaaaccttgtctggttactccgcacattacttggctttaggtttggcattattctacgttggttacatcatcttcgaagttccatctaacttgatgatggcattcattgaaccaagaatctgggtttccagaatccaattgactattggtgttgttggtgcatgtcacgctgttttgggtaccaagcatggtaacgctcaatcttacgttgcattgagattctttttgggtgttgctgaatctggtttatggccaggtttggcatactacatgtccagatggtacagaggtaaacacttaggtaaaagaattggttggtactacaccgctgcacaaattgctgcagctgcagtttctttggtttccgctggttttcaaaagatggacggtgcaagaggtttatacggttaccaatggatgttcttgatttggggtgttgttgctattgcacaagctttatctattccatggtggttgccagcagttgcttctaaggaacacagaaagtccttatcttcctttattccattgccaaagtggatgaagactttgtccccacaaagaattggtttcttaaccccagctgataagtctttgcattccagatacattgcagaaatgaacgttggtaaaagatggcaatggtctgatttgttaaagtcctgtttggacttaagagtttggccattcatcttgatgtacttcggtatcgttggtgttggtaacggtatcttcaactactgtactttgatcatcgaagaaatcaacccatctttctccggtatcgatatttctttgttgaacgctccaatttggttagcagacgctttgggtattgttactgttatgccattgtacgatagattccataagaagttctctttctttaccggttcctgtttgatcatcattgctggtttggcagttgctaactacgcaccaagagcttggtctagatacggtggtttgttaatgattggttttggtttgggtccaaccgttccaatttgtatggcatggtgttctgcatccatggctaagacttacggtgacgttggtgttgcttcttccttggcattagttaccggtttaggtaacttgggttctgttgttactacctacgctttatactccggttggccaggtgatccaactttcagaaagtctaacgacgtttgtattgctttgattggtgtttccatcatcgcatgtggtatcgaattcttgttggataagaccggtttcggtcaatttaacgcatctttcaacaaccacgatcatgaagttgaagacgaacaagaaatgactgacatcaagccagcattgccatcctcccaacaagcagacgcataaatcactttctgtcaattgtcttaat

SEQ ID NO: 4 - DNA, 3638 bp, Aspergillus oryzae
  source 1..3638: mol_type = other DNA
caaaacacacaaacaaacacaattacaaaaaatggctgcaccattcagacaaccagaagaagctgttgatgacactgaattcattgatgaccaccatgaacacttgagagataccgttcaccatagattgagagcaaactcttccattatgcacttccaaaagattttagttgctaacagaggtgaaatcccaatcagaatttttagaactgcacatgaattgtccttacaaaccgttgctatctactcccatgaagacagattgtctatgcacagacaaaaggcagatgaagcttacatgattggtcacagaggtcaatacactccagttggtgcatacttagctggtgacgaaattattaagatcgcattggaacatggtgttcaattgattcacccaggttacggtttcttgtctgaaaacgcagattttgctagaaaggttgaaaacgctggtattgttttcgttggtccaactccagataccattgactccttaggtgacaaggtttctgcaagaagattggctattaagtgtgaagttccagttgttccaggtaccgaaggtccagttgaaagatacgaagaagttaaggctttcactgatacctacggtttcccaatcattattaaggctgcatttggtggtggtggtagaggtatgagagttgttagagatcaagcagaattgagagattctttcgaaagagctacttctgaagcaagatccgcttttggtaacggtaccgttttcgttgaaagatttttagacaagccaaagcatattgaagttcaattgttgggtgactcccatggtaacgttgttcacttgttcgaaagagactgttctgttcaaagaagacaccaaaaggttgttgaagttgctccagcaaaggatttgccagcagatgttagagacagaattttagctgacgctgttaagttggctaagtctgttaactacagaaacgcaggtactgctgaattcttggttgatcaacaaaacagacattacttcatcgaaattaacccaagaattcaagttgaacacactatcaccgaagaaatcactggtatcgatattgttgctgcacaaatccaaattgctgcaggtgcttccttggaacaattgggtttaacccaagacagaatttctgcaagaggtttcgctattcaatgtagaattactaccgaagacccagcaaagggtttttccccagatactggtaaaattgaagtttacagatctgctggtggtaacggtgttagattagatggtggtaacggtttcgctggtgcaattattaccccacattacgactccatgttggttaagtgtacttgtagaggttctacctacgaaattgcaagaagaaaggttgttagagctttggttgaattcagaatcagaggtgttaagactaacattccattcttgacctctttgttatcccacccaacttttgttgatggtaactgttggactaccttcattgatgacaccccagaattgttttctttagttggttcccaaaacagagcacaaaagttgttagcttacttaggtgacgttgctgttaacggttcttccattaagggtcaaattggtgaaccaaagttgaagggtgacgttattaagccaaagttattcgacgcagaaggtaaaccattggatgtttccgctccatgtaccaagggttggaagcaaattttagatagagaaggtccagctgcatttgctaaggcagttagagcaaacaagggttgtttgattatggacactacctggagagatgcacatcaatctttgttagctactagagttagaaccatcgatttgttgaacattgctcacgaaacttcttacgcatactccaacgcttactctttagaatgttggggtggtgcaaccttcgacgttgctatgagatttttatacgaagatccatgggacagattgagaaagatgagaaaggcagttccaaacattccattccaaatgttgttaagaggtgcaaacggtgttgcttactcttccttgccagataacgcaatctaccatttttgtaagcaagctaagaagtgtggtgttgacattttcagagttttcgatgctttgaacgatgttgaccaattggaagttggtattaaggcagttcatgctgcagaaggtgttgttgaagctactatgtgttactccggtgacatgttgaacccacacaagaagtacaacttagaatactacatggcattggttgataagattgttgctatgaagccacacattttaggtattaaggacatggcaggtgttttgaagccacaagctgcaagattgttggttggttctatcagacaaagatacccagacttgccaattcacgttcatactcacgattccgcaggtaccggtgttgcttctatgattgcttgtgcacaagctggtgcagatgctgttgacgctgcaactgattctatgtccggtatgacctctcaaccatccattggtgcaattttggcttccttagaaggtaccgaacaagatccaggtttgaacttagcacatgttagagctattgactcctactgggcacaattaagattgttatactctccattcgaagctggtttgactggtccagacccagaagtttacgaacacgaaattccaggtggtcaattgaccaacttaatcttccaagcttctcaattgggtttaggtcaacaatgggcagaaactaagaaggcttacgaagctgcaaacgacttgttaggtgacattgttaaggttactccaacctccaaggttgttggtgacttggcacaattcatggtttctaacaagttgaccccagaagacgttgttgaaagagctggtgaattagatttcccaggttccgttttggaatttttagaaggtttgatgggtcaaccattcggtggttttccagaaccattaagatctagagcattgagagatagaagaaagttggaaaagaggccaggtttgtacttagaaccattggacttagctaagattaagtcccaaatcagagaaaagttcggtgctgcaactgaatacgatgttgcatcttacgctatgtacccaaaggtttttgaagactacaagaagttcgttcaaaagtttggtgacttgtccgttttgccaaccagatacttcttagcaaagccagaaatcggtgaagaattccatgttgaattggaaaagggtaaagttttgatcttaaagttgttggctattggtccattgtctgaacaaactggtcaaagagaagttttctacgaagttaacggtgaagttagacaagttgcagttgatgacaacaaggcttccgttgataacacctctagaccaaaggcagatgttggtgactcttcccaagttggtgctccaatgtccggtgttgttgttgaaattagagttcatgacggtttagaagttaagaagggtgacccattagcagttttgtctgctatgaagatggaaatggttatttccgcaccacactctggtaaagtttcttccttgttagttaaggaaggtgactctgttgacggtcaagatttggtttgtaagattgttaaggcttaaatcactttctgtcaattgtcttaat

SEQ ID NO: 5 - protein, 1180 aa, Pichia kudriavzevii
MSTVEDHSSLHKLRKESEILSNANKILVANRGEIPIRIFRSAHELSMHTVAIYSHEDRLSMHRLKADEAYAIGKTGQYSPVQAYLQIDEIIKIAKEHDVSMIHPGYGFLSENSEFAKKVEESGMIWVGPPAEVIDSVGDKVSARNLAIKCDVPVVPGTDGPIEDIEQAKQFVEQYGYPVIIKAAFGGGGRGMRVVREGDDIVDAFQRASSEAKSAFGNGTCFIERFLDKPKHIEVQLLADNYGNTIHLFERDCSVQRRHQKVVEIAPAKTLPVEVRNAILKDAVTLAKTANYRNAGTAEFLVDSQNRHYFIEINPRIQVEHTITEEITGVDIVAAQIQIAAGASLEQLGLLQNKITTRGFAIQCRITTEDPAKNFAPDTGKIEVYRSAGGNGVRLDGGNGFAGAVISPHYDSMLVKCSTSGSNYEIARRKMIRALVEFRIRGVKTNIPFLLALLTHPVFISGDCWTTFIDDTPSLFEMVSSKNRAQKLLAYIGDLCVNGSSIKGQIGFPKLNKEAEIPDLLDPNDEVIDVSKPSTNGLRPYLLKYGPDAFSKKVRGFDGCMIMDTTWRDAHQSLLATRVRTIDLLRIAPTTSHALQNAFALECWGGATFDVAMRFLYEDPWERLRQLRKAVPNIPFQMLLRGANGVAYSSLPDNAIDHFVKQAKDNGVDIFRVFDALNDLEQLKVGVDAVKKAGGVVEATVCYSGDMLIPGKKYNLDYYLETVGKIVEMGTHILGIKDMAGTLKPKAAKLLIGSIRSKYPDLVIHVHTHDSAGTGISTYVACALAGADIVDCAINSMSGLTSQPSMSAFIAALDGDIETGVPEHFARQLDAYWAEMRLLYSCFEADLKGPDPEVYKHEIPGGQLTNLIFQAQQVGLGEQWEETKKKYEDANMLLGDIVKVTPTSKVVGDLAQFMVSNKLEKEDVEKLANELDFPDSVLDFFEGLMGTPYGGFPEPLRTNVISGKRRKLKGRPGLELEPFNLEEIRENLVSRFGPGITECDVASYNMYPKVYEQYRKVVEKYGDLSVLPTKAFLAPPTIGEEVHVEIEQGKTLIIKLLAISDLSKSHGTREVYFELNGEMRKVTIEDKTAAIETVTRAKADGHNPNEVGAPMAGVVVEVRVKHGTEVKKGDPLAVLSAMKMEMVISAPVSGRVGEVFVNEGDSVDMGDLLVKIAKDEAPAA

SEQ ID NO: 6 - protein, 560 aa, Pichia kudriavzevii
MAPTAVDIHNEYKQNVSNEQEIPFNKTERKSSIASKLGLNPDAKIHYNSAVPILYEDGLKEKGTTISSSGALIAFSGSKTGRSPKDKRIVDEETSTDNIWWGPVNKKVDENTWNISKSRAIDYLRTREKVYIIDAFAGWDPRYRIKVRIVCARAYHALFMKNMLIRPTTEELKNFGEPDFTIWNAGQFPANVYTKGMTSSTSVEINFKSMEMVILGTEYAGEMKKGIFTVMFYLMPIRHKVLTLHSSANQGKKDGDVTLFFGLSGTGKTTLSADPHRELIGDDEHCWSDHGVFNIEGGCYAKCLDLSAEREPEIFNAIRFGSVLENVVYDPVDRTVDYSAANVTENTRCAYPIDFIPSAKIPCLADSHPKNIVLLTCDARGVLPPVSKLTNAQVMYHFISGYTSKMAGTEVGVTEPEATFSACFGQPFLVLHPMKYAQQLSDKMAEHSSTAWLLNTGWTGQSYVKGGKRCPLKYTRAILDAIHSGELAKQEFETYPTFGLQVPKTCPGVPESVLNPSKHWATGEADFKAEVTNLAKLFAENFEKYSAECTAEVVAAGPAL

SEQ ID NO: 7 - DNA, 1675 bp, Escherichia coli
  source 1..1675: mol_type = other DNA
catataaccccctccaaccaaacaatgagagttaacaacggtttgactccacaagaattagaagcttacggtatttctgacgttcacgatattgtttacaacccatcctacgacttgttataccaagaagaattggatccatctttaactggttacgaaagaggtgttttgaccaacttaggtgctgttgcagttgacactggtatttttaccggtagatccccaaaggataagtacattgttagagatgacactaccagagacaccttctggtgggcagataagggtaaaggtaaaaacgataacaagccattatctccagaaacttggcaacacttgaagggtttagttaccagacaattgtccggtaaaagattatttgttgttgacgctttctgtggtgcaaacccagatactagattgtctgttagattcatcaccgaagttgcttggcaagcacatttcgttaagaacatgttcatcagaccatccgacgaagaattagctggtttcaagccagattttattgttatgaacggtgcaaagtgtactaacccacaatggaaggaacaaggtttgaactctgaaaacttcgttgctttcaacttgactgaaagaatgcaattgattggtggtacctggtacggtggtgaaatgaagaagggtatgttctccatgatgaactacttgttaccattaaagggtattgcttctatgcactgttccgcaaacgttggtgaaaagggtgacgttgcagttttctttggtttgtctggtactggtaaaactaccttatccaccgatccaaagagaagattgattggtgatgacgaacatggttgggatgacgatggtgttttcaactttgaaggtggttgttacgctaagaccattaagttgtctaaggaagcagaaccagaaatttacaacgctattagaagagacgcattgttagaaaacgttactgttagagaagacggtaccattgattttgacgatggttctaagactgaaaacaccagagtttcctacccaatttaccacattgataacattgttaagccagtttccaaggctggtcatgcaactaaggttattttcttgaccgctgacgcattcggtgttttgccaccagtttctagattaactgctgatcaaacccaataccacttcttgtccggttttactgctaagttagcaggtactgaaagaggtattaccgaaccaactccaaccttctctgcttgttttggtgctgcattcttgtccttacatccaacccaatacgcagaagttttagttaagagaatgcaagctgcaggtgctcaagcatacttggttaacactggttggaacggtaccggtaaaagaatttctatcaaggacactagagctatcattgatgcaattttgaacggttccttagataacgctgaaacttttaccttgccaatgttcaacttagcaattccaactgaattaccaggtgttgacaccaagattttggatccaagaaacacttacgcttctccagaacaatggcaagaaaaggctgaaaccttggcaaagttgttcatcgacaacttcgataagtacactgataccccagcaggtgctgcattggttgctgcaggtccaaagttataagtggattaggttactgctctttcttttg

SEQ ID NO: 8 - DNA, 2704 bp, Escherichia coli
  source 1..2704: mol_type = other DNA
catataaccccctccaaccaaacaatgaacgaacaatactctgctttgagatctaacgtttccatgttgggtaaagttttaggtgaaaccattaaggacgcattgggtgaacacatcttggaaagagttgaaactatcagaaagttgtccaagtcttccagagctggtaacgacgcaaacagacaagaattgttgactaccttgcaaaacttatctaacgatgaattgttgccagttgctagagcattctcccaatttttgaacttagctaacaccgcagaacaataccattctatttccccaaagggtgaagctgcatctaacccagaagttattgctagaaccttgagaaagttaaagaaccaaccagaattgtccgaagatactattaagaaggctgttgaatctttgtccttggaattggttttgactgcacacccaactgaaatcaccagaagaactttgatccataagatggttgaagttaacgcttgtttgaagcaattagataacaaggacattgcagattacgaacacaaccaattgatgagaagattgagacaattgatcgcacaatcttggcataccgacgaaattagaaagttaagaccatccccagttgatgaggctaagtggggtttcgcagttgttgaaaactctttatggcaaggtgttccaaactacttgagagaattgaacgaacaattggaagaaaacttaggttacaagttgccagttgaattcgttccagttagattcacttcttggatgggtggtgacagagacggtaacccaaacgttaccgctgatattactagacacgttttgttattgtccagatggaaggcaaccgacttgtttttaaaggatattcaagttttagtttctgaattgtccatggttgaagctactccagaattattggcattggttggtgaagaaggtgctgcagaaccatacagatacttaatgaagaacttgagatccagattaatggctacccaagcatggttggaagctagattaaagggtgaagaattgccaaagccagaaggtttattgactcaaaacgaagaattgtgggaaccattatacgcttgttaccaatctttacaagcatgtggtatgggtattattgctaacggtgacttattggataccttgagaagagtcaagtgtttcggtgttccattagttagaatcgatattagacaagaatccaccagacacactgaagctttgggtgaattaactagatacttgggtattggtgactacgaatcttggtccgaagctgataagcaagcatttttgatcagagaattgaactctaaaagaccattgttgccaagaaactggcaaccatccgcagaaaccagagaagttttggacacttgtcaagttattgctgaagcaccacaaggttctattgctgcatacgttatttctatggcaaagactccatccgatgttttggctgttcacttgttgttaaaggaagcaggtattggtttcgctatgccagttgcaccattattcgaaaccttggatgacttaaacaacgctaacgacgttatgactcaattgttgaacatcgattggtacagaggtttgatccaaggtaaacaaatggttatgattggttactctgactccgctaaggatgcaggtgttatggctgcatcttgggctcaataccaagctcaagacgcattaattaagacctgtgaaaaggcaggtattgaattgactttattccacggtagaggtggttccattggtagaggtggtgctccagcacatgctgcattgttatctcaaccaccaggttccttgaagggtggtttaagagttaccgaacaaggtgaaatgattagattcaagtacggtttgccagaaattaccgtttcttccttgtctttatacactggtgctattttagaagcaaacttgttgccaccaccagaaccaaaggaatcctggagaagaattatggacgaattgtctgttatttcctgtgatttgtacagaggttacgttagagaaaacaaggatttcgttccatactttagatctgctaccccagaacaagaattgggtaaattgccattaggttctagaccagcaaagagaagaccaactggtggtgttgaatccttaagagctattccatggattttcgcatggacccaaaacagattgatgttaccagcttggttgggtgctggtactgcattacaaaaggttgttgaagacggtaaacaatctgaattggaagcaatgtgtagagattggccattcttttccactagattgggtatgttagaaatggtttttgctaaggcagacttgtggttagctgaatactacgaccaaagattggttgataaggcattgtggccattgggtaaagaattgagaaacttacaagaagaagatattaaggttgttttggctattgcaaacgactctcacttgatggctgatttgccatggattgcagaatccattcaattaagaaacatctacaccgacccattgaacgttttgcaagctgaattgttgcatagatctagacaagcagaaaaggaaggtcaagaaccagatccaagagttgaacaagctttgatggttaccattgcaggtattgctgctggtatgagaaacactggttaagtggattaggttactgctctttcttttg

SEQ ID NO: 9 - protein, 239 aa, Pichia kudriavzevii
MTKETKKIIQVLSQYATCDMSDALVKHQYKLGGSLPNLHRYSANETKTTMVGKAYTVLFAPKDDPREAISGGYIDKLPEDSVLVIGTTLNLQKKDAPFTKMTNALYGGLMSTRANYLRSRGTVVFGRVRDIDEHLELKRDVFSYGLGTAAHGPVVKMVGINVPLEVLVDGYPEPHVETINPGDIIMGDDNGVVRVADSEELSSIMEYIPKRVQADTLVKEDILNGLECTPAQKKRRAGL

SEQ ID NO: 10 - protein, 575 aa, Pichia kudriavzevii
MTDKISLGTYLFEKLKEAGSYSIFGVPGDFNLALLDHVKEVEGIRWVGNANELNAGYEADGYARINGFASLITTFGVGELSAVNAIAGSYAEHVPLIHIVGMPSLSAMKNNLLLHHTLGDTRFDNFTEMSKKISAKVEIVYDLESAPKLINNLIETAYHTKRPVYLGLPSNFADELVPAALVKENKLHLEEPLNNPVAEEEFIHNVVEMVKKAEKPIILVDACAARHNISKEVRELAKLTKFPVFTTPMGKSTVDEDDEEFFGLYLGSLSAPDVKDIVGPTDCILSLGGLPSDFNTGSFSYGYTTKNVVEFHSNYCKFKSATYENLMMKGAVQRLISELKNIKYSNVSTLSPPKSKFAYESAKVAPEGIITQDYLWKRLSYFLKPRDIIVTETGTSSFGVLATHLPRDSKSISQVLWGSIGFSLPAAVGAAFAAEDAHKQTGEQERRTVLFIGDGSLQLTVQSISDAARWNIKPYIFILNNRGYTIEKLIHGRHEDYNQIQPWDHQLLLKLFADKTQYENHVVKSAKDLDALMKDEAFNKEDKIRVIELFLDEFDAPEILVAQAKLSDEINSKAA

SEQ ID NO: 11 - protein, 415 aa, Pichia kudriavzevii
MFLISKSLHFTRSFSNTIKTLNRSNIKMVSPAERLSTIASTIKPNRKDSTSLQPEDYPEHPFKVTVVGSGNWGCTIAKVIAENTVERPRQFQRDVNMWVYEELIEGEKLTEIINTKHENVKYLPGIKLPVNVVAVPDIVEACAGSDLIVFNIPHQFLPRILSQLKGKVNPKARAISCLKGLDVNPNGCKLLSTVITEELGIYCGALSGANLAPEVAQCKWSETTVAYTIPDDFRGKGKDIDHQILKSLFHRPYFHVRVISDVAGISIAGALKNVVAMAAGFVEGLGWGDNAKAAVMRIGLVETIQFAKTFFDGCHAATFTHESAGVADLITTCAGGRNVRVGRYMAQHSVSATEAEEKLLNGQSCQGIHTTREVYEFLSNMGRTDEFPLFTTTYRIIYENFPIEKLPECLEPVED

SEQ ID NO: 12 - protein, 603 aa, Pichia kudriavzevii
MTKDCCEVTKIPVGEEAKVTVPRSTRLSATGPVECDLSGFQVLNSPLFNKGTAFTIAEREAFGLNGLLPPVVNTLEEQVERSYKQLHFLKTPLAKNDFCTSLRLQNKVLFYRLVKEHIKELIPIVYTPTEGDAIIAYSDRFRKPEGLFLDITRPNEIDQRLEQFGEDKDVDYIVITDSEGILGIGDQGVGGVRITIAKAALMTVCAGLHPGRVVSCVLDVGTNNVKLLEDDLYLGNRFPRVRGKEYDDFVNKTIRAMKKRFPSAVIHFEDFGVTTARPVLERFRDEIPCFNDDIQGTGAVVMASMAAALKLTHRNLLDSKVLIYGAGSAGLGIADQIVNHMVSHGATKEEARRKIYCMDRYGLILKGMTSNSPAQEDYAHDPKDWENISTTSLVDVIEKVKPTTLVGCSTQAGAFNEEVIKTMYKHNPRPMIFPLSNPTRLHECFPEDALKWTDFNALVATGSPFPPVEGHVISENNNCFAFPGIGLGAVLARTTRISDNMISAAVDELASLSPAQKDPKLGLLPPIEEIDETSARIATAVILKAVEEGFARVEEEDSPLGGKVKIPREFDPCLRWVKEQMWHPIYRPMIKVAHSDNIHTHQY

SEQ ID NO: 13 - protein, 262 aa, Pichia kudriavzevii
MASYKERSESHTSPVARRLFSIMEEKKSNLCASLDITETEKLLSILDTIGPYICLVKTHIDIVSDFTYEGTVLPLKELAKKHNFMIFEDRKFADIGNTVKNQYKSGVFRIAEWADITNAHGVTGAGIVSGLKEAAQETTSEPRGLLMLAELSSKGSLAYGEYTEKTVEIAKSDKEFVIGFIAQHDMGGREEGFDWIIMTPGVGLDDKGDALGQQYRTVDEVVKTGTDIIIVGRGLYGQGRDPVEQAKRYQQAGWNAYLNRFK

SEQ ID NO: 14 - protein, 539 aa, Pichia kudriavzevii
MTLHKNSNEGVQASGFELQDNLDVPHSNASFQSFKSDEAEQAHNNEHLMEKPQFNKATISNYCKTRFTELFPTKQSMAANKHLLNPLPGLRMIGFKQWLLILSGFLAWTWDAYDFFSISLNTVQLAKDFDKTVKDITWGITVVLMLRSVGGFFFGYLGDKYGRKWPLIANLMCVCFLEIGTGFIKNYSQFLGVRAVFGIMLGGVYGNAAATALDDCPAEARGFISGFLQQGYAFGYLLAVVFKRAIADNSPHRWRAMFWFGAGVCFLICCFRAVLPETKAFQRNKEIERYNEEHGIHQRSFKEKATTSLKIYWLMIIYMVLLMAGFNFMSHGSQDLYPTLLTVRYNFSDNATTVTNCVANIGAITGGIIIGHFSNFIGRRLSIIICCIIGGALIYPWAFVDNANINAGAFFLQFFVQGAWGVVPVHLSELAPPDFKAFVVGIAYQLGNLASSASSTIETTIGVHFPMTSPGGEPIFDYAKVMAIFVGCVFAYVLLITFIGPERKSVSFEEPVDEDIEINEKIKHNEEIEAGSNLGTSRA

SEQ ID NO: 15 - protein, 523 aa, Pichia kudriavzevii
MSDLESQHTREELDKSEDEEIQLINESRPPKLDKETIKRYLKTRFTELLPTKQQMKQNKHLLNPLPGLRMMGRRQWLMFLSAFCAWTWDAYDFFTVSLNTVQLAKDFDKNVKDITWGITLVLMLRSVGGITFGYLGDRYGRKWPLVANLLIVCILEIGSGFIKTYRQFLGVRALFGICLGGVYGNATATALDDCPTEARGFIGGLLQQGYAFGYLLAVVFKRAIADNSSHKWRATFWFGAGISFLFALFRASLPETKAFLRKKEIERYNKEHGIYQPTFQMKIVESLKNYWLMMIYLVLFMSGFSFMSHSSQDLYPTLLTVRYSFSENKATVTNCVANIGAFIGGVFTGHISNFLGRRLTIMLICIFGGALIYPWAFIDGTGINAGVFFLQWCVQGGLGVVPSHLSELAPPDLRAFVVGISYQLGNLAASASSTIETTIGEQFPMTSPSGEPIYDYAKVMAIFVGCVFAFVLIVTLFGPERRNASFENAVTTNEEFGNSAGAVDKIEHVEECIVPKHARNQQC

SEQ ID NO: 16 - protein, 506 aa, Pichia kudriavzevii
MFNPSIGEVDPSRRSSIVTAEVAKAHIKSNQRNGPEDHLHTSNDYVGYEFELSHLRTNPNNNQTINGKVQEYNVSTIEENSEDEDHDDSVYPNGYAPLLVVFGGFLSCFTLFGIMNSVGAIESYIQVNQLANASVTAISWVFSIYMFITLFSGLIVGPLYDTFGATYLMIIGTLFTFTGLLACGSSKDIYQFVLSFGVCTGIGSGCLMFPSISVISSWFNRTKRSFYIGLIQTGGSVGGVCFPILLRYLYAKYGFVWAMRIFAFFNLGVCSVACIFVRDRINEIRELTNEPIDDRTFWEKFKNSFDIRSFKDKKFIVLTAALFMNEFSLLIVITYLASYAIANGASISESYVMITIMNVSGTFGKFIPSYFAQRYGCFNMMIIMSVSMTIECFVIWLPFGKHKGALYLFIVLFGFAYAATYSLTGATIGAITPKTKDFGKRYGSAYAIVSFGNLISLPISGAFIVNRTASDYDNMVAFAASTCALASVLFLFSRYTIVGRKLRCKI

SEQ ID NO: 17 - DNA, 601 bp, Pichia kudriavzevii
  source 1..601: mol_type = other DNA
cgatgccatattgtatgtgtattgtattaagtgtgtattgtcttaagtgtgtaagagacatttatttgtgtcaacaatagcgacgccactgaaaacctcaaatatcgtatttattaatccccttcccccaagcgcagatcgtcccgtcgatttctattgtttgggcattatcagcgacgcgacggcgacgcgacggcgataatgggcgacggtcacaagatggaacgagaaaacagtttttttcggataggactcattttccaggtgagaatggggtgaccccggggagaaaccttccgcgagtggagtgcgagtggagtgggaaatgtggcccccccccccttgtgggccatgaggttgacaaataccgtgtggcccggtgatggagtgagaaagagagggaaatgataatgggaaaacaaggagaggcccgtttcccgggatttatataaagaggtgtctctatcccagttgaagtagagatttgttgatgtagttgttccttccaataaatttgttcaatcagtacacagctaatactattattacagctactactaatactactactactattactaccacccccaacacaaacaca

SEQ ID NO: 18 - DNA, 513 bp, Pichia kudriavzevii
  source 1..513: mol_type = other DNA
ctacaacaagatgtttgttcaaggggagcaacttgtccctcgttaaataatttgtaagaaaaaacttcttccttttatctctttccttttttttttttaaaaaaactatctagtaaggaaatatacacaatttactttgtacgctgtctctctttctctatctctctctatgtctatctctccctatcgctctgtatgtatgtacattaccgtcttccccaaatggctcaacccgactgcgagaagacttcaaaacactcaattatggtctttagattttccagtacgttgttgacagataccctcactattctgtcgtcgacccccctcaccgagatgttcaattgagagtcttgcacagaatactccaacgaggactggtcagacttgaggacagggtctggtctgagagcatcacgagcaattcttgcctgttcaatagatccaaaggggatattgacctgcaccgatacggggaatggcatggattggtgggatggtatggtaatcttc

SEQ ID NO: 19 - DNA, 865 bp, Pichia kudriavzevii
  source 1..865: mol_type = other DNA
cctgttggcgtatctacatcacttcctacaaacaacaccacgaattgcgtccgtggtgacgcaactacgaatggcattgtcaatgccaatgccagtgcacatacacgtgcaagtcccaccggttccctgcccggctatggtagagacaagaaggacgataccggcatcgacatcaacagtttcaacagcaatgcgtttggcgtcgacgcgtcgatggggctgccgtatttggatttggacgggctagatttcgatatggatatggatatggatatggagatgaatttgaatttagatttgggtcttgatttggggttggaattaaaaggggataacaatgagggttttcctgttgatttaaacaatggacgtgggaggtgattgatttaacctgatccaaaaggggtatgtctattttttagagtgtgtctttgtgtcaaattatggtagaatgtgtaaagtagtataaactttcctctcaaatgacgaggtttaaaacaccccccgggtgagccgagccgagaatggggcaattgttcaatgtgaaatagaagtatcgagtgagaaacttgggtgttggccagccaaggggggggggggaaggaaaatggcgcgaatgctcaggtgagattgttttggaattgggtgaagcgaggaaatgagcgacccggaggttgtgactttagtggcggaggaggacggaggaaaagccaagagggaagtgtatataaggggagcaatttgccaccaggatagaattggatgagttataattctactgtatttattgtataatttatttctccttttatatcaaacacattacaaaacacacaaaacacacaaacaaacacaattacaaaaa

SEQ ID NO: 20 - DNA, 481 bp, Pichia kudriavzevii
  source 1..481: mol_type = other DNA
atcactttctgtcaattgtcttaattattttaatatggtatttttatttgaaatactaaagcacattttcctttccacatttaatttcttaatgaactttatttctttatgatttctagatctatatttctatttgtcaactaactagattaattttaacacttacatttcttttttaaaactatgaatcataacatgcttgatagctcttatttgttttttttttacagatcaaaaaacaccttttgtagaagtaattggtctggtttgtatgtgacattaatactattttctttggaaggccgtatacatggaactaaatattttacctaacacataaaattttatttttccaaccaaagaaaaggctgaaacggatattttcttcacgttatcgaaaaataaaagcctagttaaaattgataatgaatcctgaaacgtaatcataaatagtttagaatactagctaaatcggtatcgc

SEQ ID NO: 21 - DNA, 630 bp, Pichia kudriavzevii
  source 1..630: mol_type = other DNA
caacaacacttcgccaaagacaccctttccagggaggatccactcccaacgtctctccataatgtctctgttggcccatgtctctgtcgttgacaccgtaaccacaccaaccaacccgtccattgtactgggatggtcgtccatagacacctctccaacggggaacacctcattcgtaaaccgccaaggttaccgttcctcctgactcgccccgttgttgatgctgcgcacctgtggttgcccaacatggttgtatatcgtgtaaccacaccaacacatgtgcagcacatgtgtttaaaagagtgtcatggaggtggatcatgatggaagtggactttaccacttgggaactgtctccactcccgggaagaaaagacccggcgtatcacgcggttgcctcaatggggcaatttggaaggagaaatatagggaaaatcacgtcgctctcggacggggaagagttccagactatgaggggggggggtggtatataaagacaggagatgtccacccccagagagaggaagaagttggaactttagaagagagagataactttccccagtgtccatcaatacacaaccaaacacaaactctatatttacacatataaccccctccaaccaaaca

SEQ ID NO: 22 - DNA, 501 bp, Pichia kudriavzevii
  source 1..501: mol_type = other DNA
gtggattaggttactgctctttcttttggtaatttataatttaaacaagtttatttaatttgaaactcttatttacttagattagattttaaacttacatacttttaataactctgggatatcctatttaatataactaatagctaatttgttctttttcagttgaatcttttggcgattctctctctcccttttctgttctttaacatctttaccgtaaagtattggaataaagtaatgtttgcaattagggaggtccataaaaaaatcgacccgtcgccttttcttttattcttacccatcgcgctgctataattgcaaagttcccctgtgtttgttgtattcgtttgtatttgtagaggtgtactcaatgtcgaaatctccactgtttctgtttttgctctcaaagagaaatcaaacaatgtccttcaacgtgttcaacgacggtagagtgtcccggaaattacatcgcatctctcaactataccaaatccaaccaag

SEQ ID NO: 23 - DNA, 9052 bp, synthetic construct
  misc_feature 1..9052: note = pWSPK_backbone
  source 1..9052: mol_type = other DNA
cttaccagaataatatgcagtttgctataaaaggaacaatagatctcaccggtacgaaccgccaatcaaattcccacagcgtgatatccttttcagaagacaaaaggagcaatataaaaaatgctacattgtgttatgcctaatgggatagaaaatataactctttccattactcttctggtttttattggaacaatcactcttgcaaatttccttgactgccacgttatgaatgaagaacaattacactgagggattttaaagctgccctgtagagtgatgtccttttgttaaagtctgttacactacaacaatggttttgaaaaaaaaaacccattgagaaattaaccaaagtccgggattatcggaagagcgcaacttaataaacacatcgttacaaaatatttttttttcattaaattcatttataaacgtagggactgtaaaaattgtactagatatttagtaaaagcattagttagattcatttaaatctgtttaaataagcattccaaccagcttgttggtatcttttagcttgctctataggatctcttccttgaccgtacaaacctctaccaacaattatgatatccgttccagtctttacaacttcatcaacagttctatattgttgaccaagtgcatcacctttgtcatctaaaccaacccctggagtcataatgatccagtcaaaaccttcttctctaccgcccatatcgtgttgcgcaataaaaccaatgacaaactctttatcagatttagcaatttctactgttttttctgtatattcaccatatgctaaagaaccctttgatgataactcagcaagcattagcaaacctctaggttcactggttgtttcttgggctgcctccttcaagccagaaacaatacctgcacctgttacaccatgtgcattagtgatgtcagcccattcggcaatacggaagacaccagatttatattgatttttaacagtgttaccaatatcagcaaattttctatcttcaaaaatcataaaattatgtttcttggcaagctccttcaaaggcaacacagttccttcatacgtaaaatcagaaacaatatcgatgtgtgttttaactagacagatgtaaggaccaatagtgtccaaaatagagagaagcttttcagtttcagtaatatccaatgatgcacaaaggttagacttcttttcctccatgatggagaaaagtctcctagcaacaggggaagtgtgtgattctgatctttctttgtatgacgccatccttgacaaacaaactactttattaaagcgttgaagatctattctccagcaattaaatttgtgaagaataactggtatagagtacttcctttaaaaacatgtccgtgcaccaagaaaaaaaaaaagtttgaaaaattgtatgtcgacgaatttcagcattttcatttcaaggcgatattatgtttcactaaactcaggacaggaatatactaagaataactacaacatacacacaacataagccaagatggatcaacttaactaccaagaacaacaacaatttcaaaagatcgttgaacaaaagcaaatggctgatttcatgaggctatacacatctcttgtggacagatgtttcaacgattgtgttcaagacttcacctctgaatccttaaccagcagagaaagttcatgtctaaccaaatgtgctgaaaaatttttgaagcactctgagagagttggtacccgtttccaagaacagaaccaaaagttaatgaaccaaatgagacaatgattgccgctagacaatgtcaaccttccctgtttctcgagacgcaaaccgcctctccccgcgcgttggccgattcattaatgcagctggcacgacaggtttcccgactggaaagcgggcagtgagcgcaacgcaattaatgtgagttagctcactcattaggcaccccaggctttacactttatgcttccggctcgtatgttgtgtggaattgtgagcggataacaatttcacacaggaaacagctatgaccatgattacgccaagcttgcatgcctgcaggtcgactctagaggatcctctaatggtgtacacttgaacctggttggcccattatcacttctacaagtctggaaagaatagcctatttggttcatcttcggatccccgggtaccgagctcgaattcactggccgtcgttttacaacgtcgtgactgggaaaaccctggcgttacccaacggggggcccggtacccaattcgccctatagtgagtcgtattacgcgcgcaagaatacaacaaaagaatttgtgtttctacagatgttttcggtagaggtattgatatcgaaagaatcaacttggccatcaactacgatatgccaagtgaagcagatcagtacttgcacagagttggtagagcaggtagattcggtactaaaggtttggctgtttcctttatctctaatgaaaaggatgaagaaatcttgaacaagatccaagataggtttgatgttaagattcaagagttccctgaagaaggtgttgatccttctacttacatgaacacttaattgacattgatctgtcatagttttgtggttgttttttttttgaagttatatacatttattaatatatctttatatatatattgtccaaatccatcggaaagggtctactgtaatacaatcccatatagtagaatgtactcttatatgctgcaatgaggacttgctctggagatatcgttgataagggactaccttggcttccaacgcgttggtcaacaaactgaccttgaagtgcaaatcccgacaggcacgcgtgagatatcggaggtgaatgcacctccaaatcagacaacgcgagcaaacgacgcgtaacacaaggcttgacgcgtacgatgcagacttttcatagtgtgtcgccactgagcgggaggcgggttataaaagaaacgtgtttggcgtatcttttctcttctctggatttgttcttctacttcctttactcctcatcaaatcgtctctccctcgtcactcaccacaactagtccgacactatctgatatacccttattgctaactatggacaagaagtactccattgggctcgatatcggcacaaacagcgtcggttgggccgtcattacggacgagtacaaggtgccgagcaaaaaattcaaagttctgggcaataccgatcgccacagcataaagaagaacctcattggcgccctcctgttcgactccggggagacggccgaagccacgcggctcaaaagaacagcacggcgcagatatacccgcagaaagaatcggatctgctacctgcaggagatctttagtaatgagatggctaaggtggatgactctttcttccataggctggaggagtcctttttggtggaggaggataaaaagcacgagcgccacccaatctttggcaatatcgtggacgaggtggcgtaccatgaaaagtacccaaccatatatcatctgaggaagaagcttgtagacagtactgataaggctgacttgcggttgatctatctcgcgctggcgcatatgatcaaatttcggggacacttcctcatcgagggggacctgaacccagacaacagcgatgtcgacaaactctttatccaactggttcagacttacaatcagcttttcgaagagaacccgatcaacgcatccggagttgacgccaaagcaatcctgagcgctaggctgtccaaatcccggcggctcgaaaacctcatcgcacagctccctggggagaagaagaacggcctgtttggtaatcttatcgccctgtcactcgggctgacccccaactttaaatctaacttcgacctggccgaagatgccaagcttcaactgagcaaagacacctacgatgatgatctcgacaatctgctggcccagatcggcgaccagtacgcagacctttttttggcggcaaagaacctgtcagacgccattctgctgagtgatattctgcgagtgaacacggagatcaccaaagctccgctgagcgctagtatgatcaagcgctatgatgagcaccaccaagacttgactttgctgaaggcccttgtcagacagcaactgcctgagaagtacaaggaaattttcttcgatcagtctaaaaatggctacgccggatacattgacggcggagcaagccaggaggaattttacaaatttattaagcccatcttggaaaaaatggacggcaccgaggagctgctggtaaagcttaacagagaagatctgttgcgcaaacagcgcactttcgacaatggaagcatcccccaccagattcacctgggcgaactgcacgctatcctcaggcggcaagaggatttctacccctttttgaaagataacagggaaaagattgagaaaatcctcacatttcggataccctactatgtaggccccctcgcccggggaaattccagattcgcgtggatgactcgcaaatcagaagagaccatcactccctggaacttcgaggaagtcgtggataagggggcctctgcccagtccttcatcgaaaggatgactaactttgataaaaatctgcctaacgaaaaggtgcttcctaaacactctctgctgtacgagtacttcacagtttataacgagctcaccaaggtcaaatacgtcacagaagggatgagaaagccagcattcctgtctggagagcagaagaaagctatcgtggacctcctcttcaagacgaaccggaaagttaccgtgaaacagctcaaagaagactatttcaaaaagattgaatgtttcgactctgttgaaatcagcggagtggaggatcgcttcaacgcatccctgggaacgtatcacgatctcctgaaaatcattaaagacaaggacttcctggacaatgaggagaacgaggacattcttgaggacattgtcctcacccttacgttgtttgaagatagggagatgattgaagaacgcttgaaaacttacgctcatctcttcgacgacaaagtcatgaaacagctcaagaggcgccgatatacaggatgggggcggctgtcaagaaaactgatcaatgggatccgagacaagcagagtggaaagacaatcctggattttcttaagtccgatggatttgccaaccggaacttcatgcagttgatccatgatgactctctcacctttaaggaggacatccagaaagcacaagtttctggccagggggacagtcttcacgagcacatcgctaatcttgcaggtagcccagctatcaaaaagggaatactgcagaccgttaaggtcgtggatgaactcgtcaaagtaatgggaaggcataagcccgagaatatcgttatcgagatggcccgagagaaccaaactacccagaagggacagaagaacagtagggaaaggatgaagaggattgaagagggtataaaagaactggggtcccaaatccttaaggaacacccagttgaaaacacccagcttcagaatgagaagctctacctgtactacctgcagaacggcagggacatgtacgtggatcaggaactggacatcaatcggctctccgactacgacgtggatcatatcgtgccccagtcttttctcaaagatgattctattgataataaagtgttgacaagatccgataaaaatagagggaagagtgataacgtcccctcagaagaagttgtcaagaaaatgaaaaattattggcggcagctgctgaacgccaaactgatcacacaacggaagttcgataatctgactaaggctgaacgaggtggcctgtctgagttggataaagccggcttcatcaaaaggcagcttgttgagacacgccagatcaccaagcacgtggcccaaattctcgattcacgcatgaacaccaagtacgatgaaaatgacaaactgattcgagaggtgaaagttattactctgaagtctaagctggtctcagatttcagaaaggactttcagttttataaggtgagagagatcaacaattaccaccatgcgcatgatgcctacctgaatgcagtggtaggcactgcacttatcaaaaaatatcccaagcttgaatctgaatttgtttacggagactataaagtgtacgatgttaggaaaatgatcgcaaagtctgagcaggaaataggcaaggccaccgctaagtacttcttttacagcaatattatgaattttttcaagaccgagattacactggccaatggagagattcggaagcgaccacttatcgaaacaaacggagaaacaggagaaatcgtgtgggacaagggtagggatttcgcgacagtccggaaggtcctgtccatgccgcaggtgaacatcgttaaaaagaccgaagtacagaccggaggcttctccaaggaaagtatcctcccgaaaaggaacagcgacaagctgatcgcacgcaaaaaagattgggaccccaagaaatacggcggattcgattctcctacagtcgcttacagtgtactggttgtggccaaagtggagaaagggaagtctaaaaaactcaaaagcgtcaaggaactgctgggcatcacaatcatggagcgatcaagcttcgaaaaaaaccccatcgactttctcgaggcgaaaggatataaagaggtcaaaaaagacctcatcattaagcttcccaagtactctctctttgagcttgaaaacggccggaaacgaatgctcgctagtgcgggcgagctgcagaaaggtaacgagctggcactgccctctaaatacgttaatttcttgtatctggccagccactatgaaaagctcaaagggtctcccgaagataatgagcagaagcagctgttcgtggaacaacacaaacactaccttgatgagatcatcgagcaaataagcgaattctccaaaagagtgatcctcgccgacgctaacctcgataaggtgctttctgcttacaataagcacagggataagcccatcagggagcaggcagaaaacattatccacttgtttactctgaccaacttgggcgcgcctgcagccttcaagtacttcgacaccaccatagacagaaagcggtacacctctacaaaggaggtcctggacgccacactgattcatcagtcaattacggggctctatgaaacaagaatcgacctctctcagctcggtggagacagcagggctgaccccaagaagaagaggaaggtgtgagtgagctgatagtttcttcttttacccttatatttattaaaatactcttaataatatcccatcttacatataacgaattccattcttgtcttatattcttaatcatgtcctagaaatcaaacaaaaaaaaatgtttataatgatttttttagtgttttatacattttctgtatagaagaaaaaaaaagactattattatacttacattgtaacacaattgcaacgagtgtaatttttaggttttcgttttccccctcacagctcgattattgtcaaatcacacgacaagaaaacgtaaaagcaaaaggccaggaaccgtaaaaaggccgcgttgctggcgtttttccataggctccgcccccctgacgagcatcacaaaaatcgacgctcaagtcagaggtggcgaaacccgacaggactataaagataccaggcgtttccccctggaagctccctcgtgcgctctcctgttccgaccctgccgcttaccggatacctgtccgcctttctcccttcgggaagcgtggcgctttctcatagctcacgctgtaggtatctcagttcggtgtaggtcgttcgctccaagctgggctgtgtgcacgaaccccccgttcagcccgaccgctgcgccttatccggtaactatcgtcttgagtccaacccggtaagacacgacttatcgccactggcagcagccactggtaacaggattagcagagcgaggtatgtaggcggtgctacagagttcttgaagtggtggcctaactacggctacactagaagaacagtatttggtatctgcgctctgctgaagccagttaccttcggaaaaagagttggtagctcttgatccggcaaacaaaccaccgctggtagcggtggtttttttgtttgcaagcagcagattacgcgcagaaaaaaaggatctcaagaagatcctttgatcttttctacggggtctgacgctcagtggaacgaaaactcacgttaagggattttggtcatgagattatcaaaaaggatcttcacctagatccttttaaattaaaaatgaagttttaaatcaatctaaagtatatatgagtaaacttggtctgacagttaccaatgcttaatcagtgaggcacctatctcagcgatctgtctatttcgttcatccatagttgcctgactccccgtcgtgtagataactacgatacgggagggcttaccatctggccccagtgctgcaatgataccgcgagacccacgctcaccggctccagatttatcagcaataaaccagccagccggaagggccgagcgcagaagtggtcctgcaactttatccgcctccatccagtctattaattgttgccgggaagctagagtaagtagttcgccagttaatagtttgcgcaacgttgttgccattgctacaggcatcgtggtgtcacgctcgtcgtttggtatggcttcattcagctccggttcccaacgatcaaggcgagttacatgatcccccatgttgtgcaaaaaagcggttagctccttcggtcctccgatcgttgtcagaagtaagttggccgcagtgttatcactcatggttatggcagcactgcataattctcttactgtcatgccatccgtaagatgcttttctgtgactggtgagtactcaaccaagtcattctgagaatagtgtatgcggcgaccgagttgctcttgcccggcgtcaatacgggataataccgcgccacatagcagaactttaaaagtgctcatcattggaaaacgttcttcggggcgaaaactctcaaggatcttaccgctgttgagatc

SEQ ID NO: 24 - DNA, 25 bp, synthetic construct
  misc_feature 1..25: note = 1_UP_MCH4_F
  source 1..25: mol_type = other DNA
aactttgttgtacattaagcgagtg

SEQ ID NO: 25 - DNA, 47 bp, synthetic construct
  misc_feature 1..47: note = 1_UP_MCH4_R1
  source 1..47: mol_type = other DNA
gaagtgatgtagatacgccaacaggagcagttgataatggaaaggga

SEQ ID NO: 26 - DNA, 26 bp, synthetic construct
  misc_feature 1..26: note = 1_UP_MCH4_R2
  source 1..26: mol_type = other DNA
agcagttgataatggaaagggatagg

SEQ ID NO: 27 - DNA, 25 bp, synthetic construct
  misc_feature 1..25: note = 2_PTDH3_F
  source 1..25: mol_type = other DNA
cctgttggcgtatctacatcacttc

SEQ ID NO: 28 - DNA, 31 bp, synthetic construct
  misc_feature 1..31: note = 2_PTDH3_R
  source 1..31: mol_type = other DNA
tttttgtaattgtgtttgtttgtgtgttttg

SEQ ID NO: 29 - DNA, 59 bp, synthetic construct
  misc_feature 1..59: note = 3_SpMAE1_F
  source 1..59: mol_type = other DNA
caaaacacacaaacaaacacaattacaaaaaatgggtgaattaaaggaaatcttaaagc

SEQ ID NO: 30 - DNA, 49 bp, synthetic construct
  misc_feature 1..49: note = 3_SpMAE1_R
  source 1..49: mol_type = other DNA
attaagacaattgacagaaagtgatttagacggattcgtgttcagagga

SEQ ID NO: 31 - DNA, 25 bp, synthetic construct
  misc_feature 1..25: note = 4_TGAL2_F
  source 1..25: mol_type = other DNA
atcactttctgtcaattgtcttaat

SEQ ID NO: 32 - DNA, 24 bp, synthetic construct
  misc_feature 1..24: note = 4_TGAL2_R
  source 1..24: mol_type = other DNA
gcgataccgatttagctagtattc

SEQ ID NO: 33 - DNA, 48 bp, synthetic construct
  misc_feature 1..48: note = 5_DW_MCH4_F1
  source 1..48: mol_type = other DNA
gaatactagctaaatcggtatcgctgtgtcattgtttgtatggtttag

SEQ ID NO: 34 - DNA, 51 bp, synthetic construct
  misc_feature 1..51: note = 5_DW_MCH4_F2
  source 1..51: mol_type = other DNA
ctatccctttccattatcaactgcttgtcattgtttgtatggtttaggact

SEQ ID NO: 35 - DNA, 25 bp, synthetic construct
  misc_feature 1..25: note = 5_DW_MCH4_R
  source 1..25: mol_type = other DNA
gtcaacaaatctgacatccaatatc

SEQ ID NO: 36 - DNA, 26 bp, synthetic construct
  misc_feature 1..26: note = pWSPK-F
  source 1..26: mol_type = other DNA
cttaccagaataatatgcagtttgct

SEQ ID NO: 37 - DNA, 25 bp, synthetic construct
  misc_feature 1..25: note = pWSPK-R
  source 1..25: mol_type = other DNA
gatctcaacagcggtaagatccttg

SEQ ID NO: 38 - DNA, 25 bp, synthetic construct
  misc_feature 1..25: note = sgRNA-1F
  source 1..25: mol_type = other DNA
caaggatcttaccgctgttgagatc

SEQ ID NO: 39 - DNA, 65 bp, synthetic construct
  misc_feature 1..65: note = MCH4_sgRNA-1R
  source 1..65: mol_type = other DNA
aacttgctatttctagctctaaaactggctacttctgcggtaacatgcgcaagcccggaatcgaa

SEQ ID NO: 40 - DNA, 34 bp, synthetic construct
  misc_feature 1..34: note = sgRNA-2F
  source 1..34: mol_type = other DNA
gttttagagctagaaatagcaagttaaaataagg

SEQ ID NO: 41 - DNA, 26 bp, synthetic construct
  misc_feature 1..26: note = sgRNA-2R
  source 1..26: mol_type = other DNA
agcaaactgcatattattctggtaag

SEQ ID NO: 42 - DNA, 26 bp, synthetic construct
  misc_feature 1..26: note = 1_UP_2365_F
  source 1..26: mol_type = other DNA
ggtgtccactcatatacttcattttc

SEQ ID NO: 43 - DNA, 50 bp, synthetic construct
  misc_feature 1..50: note = 1_UP_2365_R1
  source 1..50: mol_type = other DNA
acaatacacatacaatatggcatcgctgaatactatcgaatcttgccaac

SEQ ID NO: 44 - DNA, 25 bp, synthetic construct
  misc_feature 1..25: note = 1_UP_2365_R2
  source 1..25: mol_type = other DNA
ctgaatactatcgaatcttgccaac

SEQ ID NO: 45 - DNA, 25 bp, synthetic construct
  misc_feature 1..25: note = 2_PFBA1_F
  source 1..25: mol_type = other DNA
cgatgccatattgtatgtgtattgt

SEQ ID NO: 46 - DNA, 23 bp, synthetic construct
  misc_feature 1..23: note = 2_PFBA1_R
  source 1..23: mol_type = other DNA
tgtgtttgtgttgggggtggtag

SEQ ID NO: 47 - DNA, 49 bp, synthetic construct
  misc_feature 1..49: note = 3_SbMDH_F
  source 1..49: mol_type = other DNA
actaccacccccaacacaaacacaatgggtttgtctaccgcatactctc

SEQ ID NO: 48 - DNA, 49 bp, synthetic construct
  misc_feature 1..49: note = 3_SbMDH_R
  source 1..49: mol_type = other DNA
cccttgaacaaacatcttgttgtagttaaacttcacctggcaacatagt

SEQ ID NO: 49 - DNA, 24 bp, synthetic construct
  misc_feature 1..24: note = 4_TINO1_F
  source 1..24: mol_type = other DNA
ctacaacaagatgtttgttcaagg

SEQ ID NO: 50 - DNA, 23 bp, synthetic construct
  misc_feature 1..23: note = 4_TINO1_R
  source 1..23: mol_type = other DNA
gaagattaccataccatcccacc

SEQ ID NO: 51 - DNA, 52 bp, synthetic construct
  misc_feature 1..52: note = 5_DW_2365_F1
  source 1..52: mol_type = other DNA
gattggtgggatggtatggtaatcttcgatgagcatctagagttgaagaggg

SEQ ID NO: 52 - DNA, 50 bp, synthetic construct
  misc_feature 1..50: note = 5_DW_2365_F2
  source 1..50: mol_type = other DNA
gttggcaagattcgatagtattcaggatgagcatctagagttgaagaggg

SEQ ID NO: 53 - DNA, 24 bp, synthetic construct
  misc_feature 1..24: note = 5_DW_2365_R
  source 1..24: mol_type = other DNA
ccgacttgtacgaatttgttcctc

SEQ ID NO: 54 - DNA, 65 bp, synthetic construct
  misc_feature 1..65: note = 2365_sgRNA-1R
  source 1..65: mol_type = other DNA
aacttgctatttctagctctaaaacctctcggatcatcctttggctgcgcaagcccggaatcgaa

SEQ ID NO: 55 - DNA, 28 bp, synthetic construct
  misc_feature 1..28: note = PDC1_1F
  source 1..28: mol_type = other DNA
ccgtatcttattgtatcctatcctattc

SEQ ID NO: 56 - DNA, 54 bp, synthetic construct
  misc_feature 1..54: note = PDC1_1R
  source 1..54: mol_type = other DNA
atgttcattttacattcagatgtcaatttttatgttttgctgtgttttgtttta

SEQ ID NO: 57 - DNA, 39 bp, synthetic construct
  misc_feature 1..39: note = PDC1_2F
  source 1..39: mol_type = other DNA
acataaaaattgacatctgaatgtaaaatgaacattaaa

SEQ ID NO: 58 - DNA, 24 bp, synthetic construct
  misc_feature 1..24: note = PDC1_2R
  source 1..24: mol_type = other DNA
gttgaagtcaacgaagatggtgag

SEQ ID NO: 59 - DNA, 65 bp, synthetic construct
  misc_feature 1..65: note = PDC1_sgRNA-1R
  source 1..65: mol_type = other DNA
aacttgctatttctagctctaaaacgcattcaactcgttagcgtttgcgcaagcccggaatcgaa

SEQ ID NO: 60 - DNA, 27 bp, synthetic construct
  misc_feature 1..27: note = GPD1_1F
  source 1..27: mol_type = other DNA
ctctacaagagaggaaacacactacag

SEQ ID NO: 61 - DNA, 34 bp, synthetic construct
  misc_feature 1..34: note = GPD1_1R
  source 1..34: mol_type = other DNA
aaaataaatttaaaataaacgatatcaaaattca

SEQ ID NO: 62 - DNA, 59 bp, synthetic construct
  misc_feature 1..59: note = GPD1_2F
  source 1..59: mol_type = other DNA
gaattttgatatcgtttattttaaatttattttataacctcaaggagaactttggcatt

SEQ ID NO: 63 - DNA, 27 bp, synthetic construct
  misc_feature 1..27: note = GPD1_2R
  source 1..27: mol_type = other DNA
gaaatctatgcaaaccactctctcctg

SEQ ID NO: 64 - DNA, 65 bp, synthetic construct
  misc_feature 1..65: note = GPD1_sgRNA-1R
  source 1..65: mol_type = other DNA
aacttgctatttctagctctaaaacgcagattcatgagtaaaggttgcgcaagcccggaatcgaa

SEQ ID NO: 65 - DNA, 26 bp, synthetic construct
  misc_feature 1..26: note = 1_JEN2-2_F
  source 1..26: mol_type = other DNA
ccttggaccaaccaataacctgattc

SEQ ID NO: 66 - DNA, 53 bp, synthetic construct
  misc_feature 1..53: note = 1_JEN2-2_R1
  source 1..53: mol_type = other DNA
ggtgtctttggcgaagtgttgttgttgctatcttttggtattgtgcataatca

SEQ ID NO: 67 - DNA, 29 bp, synthetic construct
  misc_feature 1..29: note = 1_JEN2-2_R2
  source 1..29: mol_type = other DNA
ttgctatcttttggtattgtgcataatca

SEQ ID NO: 68 - DNA, 23 bp, synthetic construct
  misc_feature 1..23: note = 2_PENO1_F
  source 1..23: mol_type = other DNA
caacaacacttcgccaaagacac

SEQ ID NO: 69 - DNA, 24 bp, synthetic construct
  misc_feature 1..24: note = 2_PENO1_R
  source 1..24: mol_type = other DNA
tgtttggttggagggggttatatg

SEQ ID NO: 70 - DNA, 47 bp, synthetic construct
  misc_feature 1..47: note = 3_EcPCK_F
  source 1..47: mol_type = other DNA
catataaccccctccaaccaaacaatgagagttaacaacggtttgac

SEQ ID NO: 71 - DNA, 52 bp, synthetic construct
  misc_feature 1..52: note = 3_EcPCK_R
  source 1..52: mol_type = other DNA
caaaagaaagagcagtaacctaatccacttataactttggacctgcagcaac

SEQ ID NO: 72 - DNA, 48 bp, synthetic construct
  misc_feature 1..48: note = 3_EcPPC_F
  source 1..48: mol_type = other DNA
catataaccccctccaaccaaacaatgaacgaacaatactctgctttg

SEQ ID NO: 73 - DNA, 51 bp, synthetic construct
  misc_feature 1..51: note = 3_EcPPC_R
  source 1..51: mol_type = other DNA
caaaagaaagagcagtaacctaatccacttaaccagtgtttctcataccag

SEQ ID NO: 74 - DNA, 48 bp, synthetic construct
  misc_feature 1..48: note = 3_PkPCK_F
  source 1..48: mol_type = other DNA
catataaccccctccaaccaaacaatggctccaactgctgttgatatc

SEQ ID NO: 75 - DNA, 52 bp, synthetic construct
  misc_feature 1..52: note = 3_PkPCK_R
  source 1..52: mol_type = other DNA
caaaagaaagagcagtaacctaatccacttataaagcaggaccagcagcaac

SEQ ID NO: 76 - DNA, 28 bp, synthetic construct
  misc_feature 1..28: note = 4_TSED1_F
  source 1..28: mol_type = other DNA
gtggattaggttactgctctttcttttg

SEQ ID NO: 77 - DNA, 25 bp, synthetic construct
  misc_feature 1..25: note = 4_TSED1_R
  source 1..25: mol_type = other DNA
cttggttggatttggtatagttgag

SEQ ID NO: 78 - DNA, 52 bp, synthetic construct
  misc_feature 1..52: note = 5_DW_JEN2-2_F1
  source 1..52: mol_type = other DNA
ctctcaactataccaaatccaaccaagcagaagcttccatgtatgatgtatg

SEQ ID NO: 79 - DNA, 48 bp, synthetic construct
  misc_feature 1..48: note = 5_DW_JEN2-2_F2
  source 1..48: mol_type = other DNA
tatgcacaataccaaaagatagcaacagcaatgttaaccccagaagct

SEQ ID NO: 80 - DNA, 25 bp, synthetic construct
  misc_feature 1..25: note = 5_DW_JEN2-2_R
  source 1..25: mol_type = other DNA
gcagtttctgcaagatttcacacag

SEQ ID NO: 81 - DNA, 65 bp, synthetic construct
  misc_feature 1..65: note = JEN2-2_sgRNA-1R
  source 1..65: mol_type = other DNA
aacttgctatttctagctctaaaacggcaatggattcaacaaatgtgcgcaagcccggaatcgaa

SEQ ID NO: 82 - DNA, 22 bp, synthetic construct
  misc_feature 1..22: note = 1_UP_JEN2-1_F
  source 1..22: mol_type = other DNA
gataggttcaaagccctcgtcg

SEQ ID NO: 83 - DNA, 48 bp, synthetic construct
  misc_feature 1..48: note = 1_UP_JEN2-1_R1
  source 1..48: mol_type = other DNA
gaagtgatgtagatacgccaacaggggttgtgtttcaagcacctgact

SEQ ID NO: 84 - DNA, 23 bp, synthetic construct
  misc_feature 1..23: note = 1_UP_JEN2-1_R2
  source 1..23: mol_type = other DNA
ggttgtgtttcaagcacctgact

SEQ ID NO: 85 - DNA, 57 bp, synthetic construct
  misc_feature 1..57: note = 3_PkPYC1_F
  source 1..57: mol_type = other DNA
caaaacacacaaacaaacacaattacaaaaaatgtcaactgtggaagatcactcctc

SEQ ID NO: 86 - DNA, 50 bp, synthetic construct
  misc_feature 1..50: note = 3_PkPYC1_R
  source 1..50: mol_type = other DNA
attaagacaattgacagaaagtgatttaagctgctggcgcttcatctttg

SEQ ID NO: 87 - DNA, 53 bp, synthetic construct
  misc_feature 1..53: note = 3_AoPYC_F
  source 1..53: mol_type = other DNA
caaaacacacaaacaaacacaattacaaaaaatggctgcaccattcagacaac

SEQ ID NO: 88 - DNA, 50 bp, synthetic construct
  misc_feature 1..50: note = 3_AoPYC_R
  source 1..50: mol_type = other DNA
attaagacaattgacagaaagtgatttaagccttaacaatcttacaaacc

SEQ ID NO: 89 - DNA, 49 bp, synthetic construct
  misc_feature 1..49: note = 5_DW_JEN2-1_F1
  source 1..49: mol_type = other DNA
gaatactagctaaatcggtatcgcccacacccctgtggacctgttctat

SEQ ID NO: 90 - DNA, 48 bp, synthetic construct
  misc_feature 1..48: note = 5_DW_JEN2-1_F2
  source 1..48: mol_type = other DNA
agtcaggtgcttgaaacacaaccccctgtggacctgttctatgtaaac

SEQ ID NO: 91 - DNA, 23 bp, synthetic construct
  misc_feature 1..23: note = 5_DW_JEN2-1_R
  source 1..23: mol_type = other DNA
attcctcccatttctaccccctg

SEQ ID NO: 92 - DNA, 65 bp, synthetic construct
  misc_feature 1..65: note = JEN2-1_sgRNA-1R
  source 1..65: mol_type = other DNA
aacttgctatttctagctctaaaactcaagtgttcattattgtgatgcgcaagcccggaatcgaa

SEQ ID NO: 93 - DNA, 24 bp, synthetic construct
  misc_feature 1..24: note = 1_UP_MAE1_F
  source 1..24: mol_type = other DNA
tggaagacgcactagtctcaaagg

SEQ ID NO: 94 - DNA, 51 bp, synthetic construct
  misc_feature 1..51: note = 1_UP_MAE1_R1
  source 1..51: mol_type = other DNA
gaagtgatgtagatacgccaacaggggcgtgttctttttaattattgctca

SEQ ID NO: 95 - DNA, 26 bp, synthetic construct
  misc_feature 1..26: note = 1_UP_MAE1_R2
  source 1..26: mol_type = other DNA
ggcgtgttctttttaattattgctca

SEQ ID NO: 96 - DNA, 54 bp, synthetic construct
  misc_feature 1..54: note = 3_SpVHT1_F
  source 1..54: mol_type = other DNA
caaaacacacaaacaaacacaattacaaaaaatggcatccgaatggccagaaac

SEQ ID NO: 97 - DNA, 50 bp, synthetic construct
  misc_feature 1..50: note = 3_SpVHT1_R
  source 1..50: mol_type = other DNA
attaagacaattgacagaaagtgatttatgcgtctgcttgttgggaggat

SEQ ID NO: 98 - DNA, 50 bp, synthetic construct
  misc_feature 1..50: note = 5_DW_MAE1_F1
  source 1..50: mol_type = other DNA
gaatactagctaaatcggtatcgctggacacatacacattatcaaatgca

SEQ ID NO: 99 - DNA, 50 bp, synthetic construct
  misc_feature 1..50: note = 5_DW_MAE1_F2
  source 1..50: mol_type = other DNA
gagcaataattaaaaagaacacgcctggacacatacacattatcaaatgc

SEQ ID NO: 100 - DNA, 24 bp, synthetic construct
  misc_feature 1..24: note = 5_DW_MAE1_R
  source 1..24: mol_type = other DNA
gctaagcacaccggccttggaaac

SEQ ID NO: 101 - DNA, 65 bp, synthetic construct
  misc_feature 1..65: note = MAE1_sgRNA-1R
  source 1..65: mol_type = other DNA
aacttgctatttctagctctaaaaccctctcccactggaatcttttgcgcaagcccggaatcgaa

SEQ ID NO: 102 - DNA, 546 bp, synthetic construct
  misc_feature 1..546: note = PDC1_sgRNA_1
  source 1..546: mol_type = other DNA
caaggatcttaccgctgttgagatccagttcgatgtaacccactcgtgcacccaactgatcttcagcatcttttactttcaccagcgtttctgggtgagcaaaaacaggaaggcaaaatgccgcaaaaaagggaataagggcgacacggaaatgttgaatactcatactcttcctttttcaatattattgaagcatttatcagggttattgtctcatgagcggatacatatttgaatgtatttagaaaaataaacaaataggggttccgcgcacatttccccgaaaagtgccacctgacgtcccaatgattttaactttctccttgaacttctgtctaaccttctacaatcttcttcaagcttctatttgatttctcaaatcaaagatagaaaaagagtattttgtctaatctctaaaaaatcaatacaagcgcaagtggtttagtggtaaaattcaacgttgccatcgttgagcccctggttcgattccgggcttgcgcaaacgctaacgagttgaatgcgttttagagctagaaatagcaagtt

SEQ ID NO: 103 - DNA, 500 bp, synthetic construct
  misc_feature 1..500: note = sgRNA_2
  source 1..500: mol_type = other DNA
gttttagagctagaaatagcaagttaaaataaggctagtccgttatcaacttgaaaaagtggcaccgagtcggtgctttttttatcggaaagaacatgtgagcaaaaggccggttagacctagttcaaaagccaaagtgcctaattcctctagaaaatgtgtagatttcagattcgaaacccaagtttggcggcccaaaaaaaccattcaatccactcggccacgcaagtttcaaaggtggcaaaaaaaaatgcggtaataacaatcatttattaatcacgtgattgcaagagtgttaaaatgaaatttgaaaaaaaaaaggattgtcttatcttaaccacaaccacatagaggcttgggagattttgtttagcaacaaattttgagaaaaactagtactctaaaagcttcttgtctttgcaaggagagaatttacagcaaatttgtcttaacctcttttgaatttgataacttcttaccagaataatatgcagtttgct

SEQ ID NO: 104 - DNA, 789 bp, synthetic construct
  misc_feature 1..789: note = PkURA3
  source 1..789: mol_type = other DNA
atggcgtcatacaaagaaagatcagaatcacacacttcccctgttgctaggagacttttctccatcatggaggaaaagaagtctaacctttgtgcatcattggatattactgaaactgaaaagcttctctctattttggacactattggtccttacatctgtctagttaaaacacacatcgatattgtttctgattttacgtatgaaggaactgtgttgcctttgaaggagcttgccaagaaacataattttatgatttttgaagatagaaaatttgctgatattggtaacactgttaaaaatcaatataaatctggtgtcttccgtattgccgaatgggctgacatcactaatgcacatggtgtaacgggtgcaggtattgtttctggcttgaaggaggccgcccaagaaacaaccagtgaacctagaggtttgctaatgcttgctgagttatcatcaaagggttctttagcatatggtgaatatacagaaaaaacagtagaaattgctaaatctgataaagagtttgtcattggttttattgcgcaacacgatatgggcggtagagaagaaggttttgactggatcattatgactccaggggttggtttagatgacaaaggtgatgcacttggtcaacaatatagaactgttgatgaagttgtaaagactggaacggatatcataattgttggtagaggtttgtatggtcaaggaagagatcctgtagagcaagctaaaagataccaacaagctggttggaatgcttatttaaacagatttaaatga

SEQ ID NO: 105 - DNA, 632 bp, synthetic construct
  misc_feature 1..632: note = PkURA3 promoter
  source 1..632: mol_type = other DNA
ggtatagtccgtcagttatattggaagataataagaaaagaatatcaaaactatttaattagttaattgtataaactgtatgtcattataaacagggaaggttgacattgtctagcggcaatcattgtctcatttggttcattaacttttggttctgttcttggaaacgggtaccaactctctcagagtgcttcaaaaatttttcagcacatttggttagacatgaactttctctgctggttaaggattcagaggtgaagtcttgaacacaatcgttgaaacatctgtccacaagagatgtgtatagcctcatgaaatcagccatttgcttttgttcaacgatcttttgaaattgttgttgttcttggtagttaagttgatccatcttggcttatgttgtgtgtatgttgtagttattcttagtatattcctgtcctgagtttagtgaaacataatatcgccttgaaatgaaaatgctgaaattcgtcgacatacaatttttcaaactttttttttttcttggtgcacggacatgtttttaaaggaagtactctataccagttattcttcacaaatttaattgctggagaatagatcttcaacgctttaataaagtagtttgtttgtcaagg

SEQ ID NO: 106 - DNA, 493 bp, synthetic construct
  misc_feature 1..493: note = PkURA3 terminator
  source 1..493: mol_type = other DNA
ttcttacacaaagatttgatacatgtacactagtttaaataagcatgaaaagaattacacaagcaaaaaaaaaattaaatgaggtactttacgttcacctacaaccaaaaaaactagatagagtaaaatcttatgatttagaaaaagttgtttaacaaaggctttagtatgtgaatttttaatgtagcaaagcgataactaataaacataaacaaaagtatggttttctttatcagtcaaatcattatcgattgattgttccgcgtattctaagtgttttatatcattcatagttaacgattgcttttgtttattctgtattctcagcataagatagtaaaggataccggtgaacgccataattgaaaaggaagcttccatggcatgtatccccatcggatactttggtgcttgagaacctttgaaaaaatatggaccgataatgttaccaactgcataccaaactgcaacagaaacatacatgaacgtcttc

SEQ ID NO: 107 - DNA, 24 bp, synthetic construct
  misc_feature 1..24: note = 1_UP_MCH5_F
  source 1..24: mol_type = other DNA
gtgcaggaatttcaagatagtcgg

SEQ ID NO: 108 - DNA, 52 bp, synthetic construct
  misc_feature 1..52: note = 1_UP_MCH5_R1
  source 1..52: mol_type = other DNA
cttccaatataactgacggactataccccttgtgctctatctctatgttccc

SEQ ID NO: 109 - DNA, 25 bp, synthetic construct
  misc_feature 1..25: note = 1_UP_MCH5_R2
  source 1..25: mol_type = other DNA
ccttgtgctctatctctatgttccc

SEQ ID NO: 110 - DNA, 28 bp, synthetic construct
  misc_feature 1..28: note = 2_PkURA3_F
  source 1..28: mol_type = other DNA
ggtatagtccgtcagttatattggaaga

SEQ ID NO: 111 - DNA, 26 bp, synthetic construct
  misc_feature 1..26: note = 2_PkURA3_R
  source 1..26: mol_type = other DNA
gaagacgttcatgtatgtttctgttg

SEQ ID NO: 112 - DNA, 50 bp, synthetic construct
  misc_feature 1..50: note = 3_DW_MCH5_F1
  source 1..50: mol_type = other DNA
aacagaaacatacatgaacgtcttcttacatccgagtctgttgtattgcc

SEQ ID NO: 113 - DNA, 50 bp, synthetic construct
  misc_feature 1..50: note = 3_DW_MCH5_F2
  source 1..50: mol_type = other DNA
gggaacatagagatagagcacaaggttacatccgagtctgttgtattgcc

SEQ ID NO: 114 - DNA, 23 bp, synthetic construct
  misc_feature 1..23: note = 3_DW_MCH5_R
  source 1..23: mol_type = other DNA
atggggtctcctgaacatttgtg

SEQ ID NO: 115 - DNA, 65 bp, synthetic construct
  misc_feature 1..65: note = MCH5_sgRNA-1R
  source 1..65: mol_type = other DNA
aacttgctatttctagctctaaaaccgatcgcacgaactactgtttgcgcaagcccggaatcgaa